European Patent Specification EP 4 252 003 B1, published March 5, 2025. Title: ANALYTICAL METHOD FOR GLYCOCONJUGATES USING A CAPILLARY-BASED IMMUNOASSAY SYSTEM. Applicant: Janssen Pharmaceuticals, Inc. The sequence listing filed with the application follows.

SEQUENCE LISTING (3 sequences)

SEQ ID NO: 1 - skipped

SEQ ID NO: 2 - protein, 5 aa, Artificial Sequence
  optimized glycosylation consensus sequence
  VARIANT 1: Asp or Glu
  VARIANT 2: any amino acid residue except Pro
  VARIANT 4: any amino acid residue except Pro
  VARIANT 5: Ser or Thr
XXNXX

SEQ ID NO: 3 - protein, 652 aa, Artificial Sequence
  EPA carrier protein including 4 N-linked glycosylation consensus sequences
GSGGGDQNATGSGGGKLAEEAFDLWNECAKACVLDLKDGVRSSRMSVDPAIADTNGQGVLHYSMVLEGGNDALKLAIDNALSITSDGLTIRLEGGVEPNKPVRYSYTRQARGSWSLNWLVPIGHEKPSNIKVFIHELNAGNQLSHMSPIYTIEMGDELLAKLARDATFFVRAHESNEMQPTLAISHAGVSVVMAQAQPRREKRWSEWASGKVLCLLDPLDGVYNYLAQQRCNLDDTWEGKIYRVLAGNPAKHDLDIKDNNNSTPTVISHRLHFPEGGSLAALTAHQACHLPLEAFTRHRQPRGWEQLEQCGYPVQRLVALYLAARLSWNQVDQVIRNALASPGSGGDLGEAIREQPEQARLALTLAAAESERFVRQGTGNDEAGAASADVVSLTCPVAKDQNRTKGECAGPADSGDALLERNYPTGAEFLGDGGDVSFSTRGTQNWTVERLLQAHRQLEERGYVFVGYHGTFLEAAQSIVFGGVRARSQDLDAIWRGFYIAGDPALAYGYAQDQEPDARGRIRNGALLRVYVPRWSLPGFYRTGLTLAAPEAAGEVERLIGHPLPLRLDAITGPEEEGGRVTILGWPLAERTVVIPSAIPTDPRNVGGDLDPSSIPDKEQAISALPDYASQPGKPPREDLKLGSGGGDQNAT